European Patent Application EP 4 512 412 A1, published February 26, 2025. Title: 多肽及其用途. Applicant: 深圳辰扬生物科技有限公司. The sequence listing filed with the application follows.

SEQUENCE LISTING (5 sequences)

SEQ ID NO: 1 - protein, 15 aa, synthetic construct
KRSSRAFRAHLRAPL

SEQ ID NO: 2 - protein, 443 aa, Homo sapiens
MDPLNLSWYDDDLERQNWSRPFNGSDGKADRPHYNYYATLLTLLIAVIVFGNVLVCMAVSREKALQTTTNYLIVSLAVADLLVATLVMPWVVYLEVVGEWKFSRIHCDIFVTLDVMMCTASILNLCAISIDRYTAVAMPMLYNTRYSSKRRVTVMISIVWVLSFTISCPLLFGLNNADQNECIIANPAFVVYSSIVSFYVPFIVTLLVYIKIYIVLRRRRKRVNTKRSSRAFRAHLRAPLKGNCTHPEDMKLCTVIMKSNGSFPVNRRRVEAARRAQELEMEMLSSTSPPERTRYSPIPPSHHQLTLPDPSHHGLHSTPDSPAKPEKNGHAKDHPKIAKIFEIQTMPNGKTRTSLKTMSRRKLSQQKEKKATQMLAIVLGVFIICWLPFFITHILNIHCDCNIPPVLYSAFTWLGYVNSAVNPIIYTTFNIEFRKAFLKILHC

SEQ ID NO: 3 - DNA, 1525 bp, Homo sapiens
  source 1..1525: mol_type = genomic DNA
ctggccacccagtcggtccaccgccctgatggatccactgaatctgtcctggtatgatgatgatctggagaggcagaactggagccggcccttcaacgggtcagacgggaaggcggacagaccccactacaactactatgccacactgctcaccctgctcatcgctgtcatcgtcttcggcaacgtgctggtgtgcatggctgtgtcccgcgagaaggcgctgcagaccaccaccaactacctgatcgtcagcctcgcagtggccgacctcctcgtcgccacactggtcatgccctgggttgtctacctggaggtggtaggtgagtggaaattcagcaggattcactgtgacatcttcgtcactctggacgtcatgatgtgcacggcgagcatcctgaacttgtgtgccatcagcatcgacaggtacacagctgtggccatgcccatgctgtacaatacgcgctacagctccaagcgccgggtcaccgtcatgatctccatcgtctgggtcctgtccttcaccatctcctgcccactcctcttcggactcaataacgcagaccagaacgagtgcatcattgccaacccggccttcgtggtctactcctccatcgtctccttctacgtgcccttcattgtcaccctgctggtctatatcaagatctacattgtcctccgcagacgccgcaagcgagtcaacaccaaacgcagcagccgagctttcagggcccacctgagggctccactaaagggcaactgtactcaccccgaggacatgaaactctgcaccgttatcatgaagtctaatgggagtttcccagtgaacaggcggagagtggaggctgcccggcgagcccaggagctggagatggagatgctctccagcaccagcccacccgagaggacccggtacagccccatcccacccagccaccaccagctgactctccccgacccgtcccaccatggtctccacagcactcccgacagccccgccaaaccagagaagaatgggcatgccaaagaccaccccaagattgccaagatctttgagatccagaccatgcccaatggcaaaacccggacctccctcaagaccatgagccgtaggaagctctcccagcagaaggagaagaaagccactcagatgctcgccattgttctcggcgtgttcatcatctgctggctgcccttcttcatcacacacatcctgaacatacactgtgactgcaacatcccgcctgtcctgtacagcgccttcacgtggctgggctatgtcaacagcgccgtgaaccccatcatctacaccaccttcaacattgagttccgcaaggccttcctgaagatcctccactgctgactctgctgcctgcccgcacagcagcctgcttcccacctccctgcccaggccggccagcctcacccttgcgaaccgtgagcaggaaggcctgggtggatcggcctcctcttcaccccggcaggccctgcagtgttcgcttggctccatgctcctcactgcccgcac

SEQ ID NO: 4 - DNA, 45 bp, synthetic construct
  source 1..45: mol_type = other DNA
aaacgcagcagccgagctttcagggcccacctgagggctccacta

SEQ ID NO: 5 - protein, 11 aa, synthetic construct
YGRKKRRQRRR